European Patent Application EP 4 678 760 A1, published January 14, 2026. Title: MICROORGANISM HAVING INCREASED ACTIVITY OF PYRUVATE DEHYDROGENASE COMPLEX SUBUNIT E1 AND METHOD FOR PRODUCING O-ACETYLHOMOSERINE OR DERIVATIVES THEREOF USING THE SAME. Applicant: 씨제이제일제당 주식회사. Application KR. The sequence listing filed with the application follows.

SEQUENCE LISTING (35 sequences)

SEQ ID NO: 1 - protein, 922 aa, Corynebacterium glutamicum
  source 1..922: note = ATCC13869 & ATCC13032_aceE_NCgl216
MADQAKLGGKPSDDSNFAMIRDGVASYLNDSDPEETNEWMDSLDGLLQESSPERARYLMLRLLERASAKRVSLPPMTSTDYVNTIPTSMEPEFPGDEEMEKRYRRWIRWNAAIMVHRAQRPGIGVGGHISTYAGAAPLYEVGFNHFFRGKDHPGGGDQIFFQGHASPGMYARAFMEGRLSEDDLDGFRQEVSREQGGIPSYPHPHGMKDFWEFPTVSMGLGPMDAIYQARFNRYLENRGIKDTSDQHVWAFLGDGEMDEPESRGLIQQAALNNLDNLTFVVNCNLQRLDGPVRGNTKIIQELESFFRGAGWSVIKVVWGREWDELLEKDQDGALVEIMNNTSDGDYQTFKANDGAYVREHFFGRDPRTAKLVENMTDEEIWKLPRGGHDYRKVYAAYKRALETKDRPTVILAHTIKGYGLGHNFEGRNATHQMKKLTLDDLKLFRDKQGIPITDEQLEKDPYLPPYYHPGEDAPEIKYMKERRAALGGYLPERRENYDPIQVPPLDKLRSVRKGSGKQQIATTMATVRTFKELMRDKGLADRLVPIIPDEARTFGLDSWFPTLKIYNPHGQNYVPVDHDLMLSYREAPEGQILHEGINEAGSVASFIAAGTSYATHGKAMIPLYIFYSMFGFQRTGDSIWAAADQMARGFLLGATAGRTTLTGEGLQHMDGHSPVLASTNEGVETYDPSFAYEIAHLVHRGIDRMYGPGKGEDVIYYITIYNEPTPQPAEPEGLDVEGLHKGIYLYSRGEGTGHEANILASGVGMQWALKAASILEADYGVRANIYSATSWVNLARDGAARNKAQLRNPGADAGEAFVTTQLKQTSGPYVAVSDFSTDLPNQIREWVPGDYTVLGADGFGFSDTRPAARRFFNIDAESIVVAVLNSLAREGKIDVSVAAQAAEKFKLDDPTSVSVDPNAPEE

SEQ ID NO: 2 - DNA, 2769 bp, Corynebacterium glutamicum
  source 1..2769: mol_type = genomic DNA; note = ATCC13032_aceE
atggccgatcaagcaaaacttggtggcaagccctcggatgactctaacttcgcgatgatccgcgatggcgtggcatcttatttgaacgactcagatccggaggagaccaacgagtggatggattcactcgacggattactccaggagtcttctccagaacgtgctcgttacctcatgcttcgtttgcttgagcgtgcatctgcaaagcgcgtatctcttcccccaatgacgtcaaccgactacgtcaacaccattccaacctctatggaacctgaattcccaggcgatgaggaaatggagaagcgttaccgtcgttggattcgctggaacgcagccatcatggttcaccgcgctcagcgaccaggcatcggcgtcggcggacacatttccacttacgcaggcgcagcccctctgtacgaagttggcttcaaccacttcttccgcggcaaggatcacccaggcggcggcgaccagatcttcttccagggccacgcatcaccaggtatgtacgcacgtgcattcatggagggtcgcctttctgaagacgatctcgatggcttccgtcaggaagtttcccgtgagcagggtggcattccgtcctaccctcacccacacggtatgaaggacttctgggagttcccaactgtgtccatgggtcttggcccaatggatgccatttaccaggcacgtttcaaccgctacctcgaaaaccgtggcatcaaggacacctctgaccagcacgtctgggccttccttggcgacggcgaaatggacgagccagaatcacgtggtctcatccagcaggctgcactgaacaacctggacaacctgaccttcgtggttaactgcaacctgcagcgtctcgacggacctgtccgcggtaacaccaagatcatccaggaactcgagtccttcttccgtggcgcaggctggtctgtgatcaaggttgtttggggtcgcgagtgggatgaacttctggagaaggaccaggatggtgcacttgttgagatcatgaacaacacctccgatggtgactaccagaccttcaaggctaacgacggcgcatatgttcgtgagcacttcttcggacgtgacccacgcaccgcaaagctcgttgagaacatgaccgacgaagaaatctggaagcttccacgtggcggccacgattaccgcaaggtttacgcagcctacaagcgagctcttgagaccaaggatcgcccaaccgtcatccttgctcacaccattaagggctacggactcggccacaacttcgaaggccgtaacgcaacccaccagatgaagaagctgacgcttgatgatctgaagttgttccgcgacaagcagggcatcccaatcaccgatgagcagctggagaaggatccttaccttcctccttactaccacccaggtgaagacgctcctgaaatcaagtacatgaaggaacgtcgcgcagcgctcggtggctacctgccagagcgtcgtgagaactacgatccaattcaggttccaccactggataagcttcgctctgtccgtaagggctccggcaagcagcagatcgctaccaccatggcgactgttcgtaccttcaaggaactgatgcgcgataagggcttggctgatcgccttgtcccaatcattcctgatgaggcacgtaccttcggtcttgactcttggttcccaaccttgaagatctacaacccgcacggtcagaactacgtgcctgttgaccacgacctgatgctctcctaccgtgaggcacctgaaggacagatcctgcacgaaggcatcaacgaggctggttccgtggcatcgttcatcgctgcgggtacctcctacgccacccacggcaaggccatgattccgctgtacatcttctactcgatgttcggattccagcgcaccggtgactccatctgggcagcagccgatcagatggcacgtggcttcctcttgggcgctaccgcaggtcgcaccaccctgaccggtgaaggcctccagcacatggatggacactcccctgtcttggcttccaccaacgagggtgtcgagacctacgacccatcctttgcgtacgagatcgcacacctggttcaccgtggcatcgaccgcatgtacggcccaggcaagggtgaagatgttatctactacatcaccatctacaacgagccaaccccacagccagctgagccagaaggactggacgtagaaggcctgcacaagggcatctacctctactcccgcggtgaaggcaccggccatgaggcaaacatcttggcttccggtgttggtatgcagtgggctctcaaggctgcatccatccttgaggctgactacggagttcgtgccaacatttactccgctacttcttgggttaacttggctcgcgatggcgctgctcgtaacaaggcacagctgcgcaacccaggtgcagatgctggcgaggcattcgtaaccacccagctgaagcagacctccggcccatacgttgcagtgtctgacttctccactgatctgccaaaccagatccgtgaatgggtcccaggcgactacaccgttctcggtgcagatggcttcggtttctctgatacccgcccagctgctcgtcgcttcttcaacatcgacgctgagtccattgttgttgcagtgctgaactccctggcacgcgaaggcaagatcgacgtctccgttgctgctcaggctgctgagaagttcaagttggatgatcctacgagtgtttccgtagatccaaacgctcctgaggaataa

SEQ ID NO: 3 - DNA, 2769 bp, Corynebacterium glutamicum
  source 1..2769: mol_type = genomic DNA; note = ATCC13869_aceE
atggccgatcaagcaaaacttggtggtaagccctcggatgactctaacttcgcgatgatccgcgatggcgtggcatcttatttgaacgactcagatccggaggagaccaacgagtggatggattcactcgacggattactccaggagtcttctccagaacgtgctcgttacctcatgcttcgtttgcttgagcgtgcatctgcaaagcgcgtatctcttcccccaatgacgtcaaccgactacgtcaacaccattccaacctctatggaacctgaattcccaggcgatgaggaaatggagaagcgttaccgtcgttggattcgctggaacgcagccatcatggttcaccgcgctcagcgaccaggcatcggcgtcggcggacacatttccacttacgcaggcgcagcccctctgtacgaagttggcttcaaccacttcttccgcggcaaggatcacccaggcggcggcgaccagatcttcttccagggccacgcatcaccaggtatgtacgcacgtgcattcatggagggtcgcctttctgaagacgatctcgatggcttccgtcaggaagtttcccgtgagcagggtggcattccgtcctaccctcacccacacggtatgaaggacttctgggagttcccaactgtgtccatgggtcttggcccaatggatgccatttaccaggcacgtttcaaccgctacctcgaaaaccgtggcatcaaggacacctctgaccagcacgtctgggccttccttggcgacggcgaaatggacgagccagaatcacgtggtctcatccagcaggctgcactgaacaacctggacaacctgaccttcgtggttaactgcaacctgcagcgtctcgacggacctgtccgcggtaacaccaagatcatccaggaactcgagtccttcttccgtggcgcaggctggtctgtgatcaaggttgtttggggtcgcgagtgggatgaacttctggagaaggaccaggatggtgcacttgttgagatcatgaacaacacctccgatggtgactaccagaccttcaaggctaacgacggcgcatatgttcgtgagcacttcttcggacgtgacccacgcaccgcaaagctcgttgagaacatgaccgacgaagaaatctggaagctgccacgtggcggccacgattaccgcaaggtttacgcagcctacaagcgagctcttgagaccaaggatcgcccaaccgtcatccttgctcacaccattaagggctacggactcggccacaacttcgaaggccgtaacgcaacccaccagatgaagaagctgacgcttgatgatctgaagttgttccgcgacaagcagggcatcccaatcaccgatgagcagctggagaaggatccttaccttcctccttactaccacccaggtgaagacgctcctgaaatcaagtacatgaaggaacgtcgcgcagcgctcggtggctacctgccagagcgtcgtgagaactacgatccaattcaggttccaccactggataagcttcgctctgtccgtaagggctccggcaagcagcagatcgctaccactatggcgactgttcgtaccttcaaggaactgatgcgcgataagggcttggctgatcgccttgtcccaatcattcctgatgaggcacgtaccttcggtcttgactcttggttcccaaccttgaagatctacaacccgcacggtcagaactacgtgcctgttgaccacgacctgatgctctcctaccgtgaggcacctgaaggacagatcctgcacgaaggcatcaacgaggctggttccgtggcatcgttcatcgctgcgggtacctcctacgccacccacggcaaggccatgattccgctgtacatcttctactcgatgttcggattccagcgcaccggtgactccatctgggcagcagccgatcagatggcacgtggcttcctcttgggcgctaccgcaggtcgcaccaccctgaccggtgaaggcctccagcacatggatggacactcccctgtcttggcttccaccaacgagggtgtcgagacctacgacccatcctttgcgtacgagatcgcacacctggttcaccgtggcatcgaccgcatgtacggcccaggcaagggtgaagatgttatctactacatcaccatctacaacgagccaaccccacagccagctgagccagaaggactggacgtagaaggcctgcacaagggcatctacctctactcccgcggtgaaggcaccggccatgaggcaaacatcttggcttccggtgttggtatgcagtgggctctcaaggctgcatccatccttgaggctgactacggagttcgtgccaacatttactccgctacttcttgggttaacttggctcgcgatggcgctgctcgtaacaaggcacagctgcgcaacccaggtgcagatgctggcgaggcattcgtaaccacccagctgaagcagacctccggcccatacgttgcagtgtctgacttctccactgatctgccaaaccagatccgtgaatgggtcccaggcgactacaccgttctcggtgcagatggcttcggtttctctgatacccgcccagctgctcgtcgcttcttcaacatcgacgctgagtccattgttgttgcagtgctgaactccctggcacgcgaaggcaagatcgacgtctccgttgctgctcaggctgctgagaagttcaagttggatgatcctacgagtgtttccgtagatccaaacgctcctgaggaataa

SEQ ID NO: 4 - DNA, 1161 bp, Corynebacterium glutamicum
  source 1..1161: mol_type = genomic DNA; note = Ncgl2360 (metB)
ttgtcttttgacccaaacacccagggtttctccactgcatcgattcacgctgggtatgagccagacgactactacggttcgattaacaccccaatctatgcctccaccaccttcgcgcagaacgctccaaacgaactgcgcaaaggctacgagtacacccgtgtgggcaaccccaccatcgtggcattagagcagaccgtcgcagcactcgaaggcgcaaagtatggccgcgcattctcctccggcatggctgcaaccgacatcctgttccgcatcatcctcaagccgggcgatcacatcgtcctcggcaacgatgcttacggcggaacctaccgcctgatcgacaccgtattcaccgcatggggcgtcgaatacaccgttgttgatacctccgtcgtggaagaggtcaaggcagcgatcaaggacaacaccaagctgatctgggtggaaaccccaaccaacccagcacttggcatcaccgacatcgaagcagtagcaaagctcaccgaaggcaccaacgccaagctggttgttgacaacaccttcgcatccccatacctgcagcagccactaaaactcggcgcacacgcagtcctgcactccaccaccaagtacatcggaggacactccgacgttgttggcggccttgtggttaccaacgaccaggaaatggacgaagaactgctgttcatgcagggcggcatcggaccgatcccatcagttttcgatgcatacctgaccgcccgtggcctcaagacccttgcagtgcgcatggatcgccactgcgacaacgcagaaaagatcgcggaattcctggactcccgcccagaggtctccaccgtgctctacccaggtctgaagaaccacccaggccacgaagtcgcagcgaagcagatgaagcgcttcggcggcatgatctccgtccgtttcgcaggcggcgaagaagcagctaagaagttctgtacctccaccaaactgatctgtctggccgagtccctcggtggcgtggaatccctcctggagcacccagcaaccatgacccaccagtcagctgccggctctcagctcgaggttccccgcgacctcgtgcgcatctccattggtattgaagacattgaagacctgctcgcagatgtcgagcaggccctcaataacctttag

SEQ ID NO: 5 - DNA, 318 bp, synthetic construct
  source 1..318: mol_type = other DNA; note = Pcj7
agaaacatcccagcgctactaatagggagcgttgaccttccttccacggaccggtaatcggagtgcctaaaaccgcatgcggcttaggctccaagataggttctgcgcggccgggtaatgcatcttctttagcaacaagttgaggggtaggtgcaaataagaacgacatagaaatcgtctcctttctgtttttaatcaacatacaccaccacctaaaaattccccgaccagcaagttcacagtattcgggcacaatatcgttgccaaaatattgtttcggaatatcatgggatacgtacccaacgaaaggaaacactc

SEQ ID NO: 6 - DNA, 18 bp, synthetic construct
  source 1..18: mol_type = other DNA
ggcttcggagttggagcg

SEQ ID NO: 7 - DNA, 40 bp, synthetic construct
  source 1..40: mol_type = other DNA
gccaaatagtttcccgggggtagatcaactcctgtaatca

SEQ ID NO: 8 - DNA, 40 bp, synthetic construct
  source 1..40: mol_type = other DNA
caggagttgatctacccccgggaaactatttggcggcaag

SEQ ID NO: 9 - DNA, 19 bp, synthetic construct
  source 1..19: mol_type = other DNA
tcgcgtctgggtgcgcatc

SEQ ID NO: 10 - DNA, 34 bp, synthetic construct
  source 1..34: mol_type = other DNA
agaaacatcccagcgctactaatagggagcgttg

SEQ ID NO: 11 - DNA, 32 bp, synthetic construct
  source 1..32: mol_type = other DNA
atgggatacgtacccaacgaaaggaaacactc

SEQ ID NO: 12 - DNA, 42 bp, synthetic construct
  source 1..42: mol_type = other DNA
gtgaattcgagctcggtaccccactggccagcgattaacttt

SEQ ID NO: 13 - DNA, 42 bp, synthetic construct
  source 1..42: mol_type = other DNA
tagtagcgctgggatgtttctttccacacctcctgttggaat

SEQ ID NO: 14 - DNA, 40 bp, synthetic construct
  source 1..40: mol_type = other DNA
ccaacgaaaggaaacactcatggccgatcaagcaaaactt

SEQ ID NO: 15 - DNA, 42 bp, synthetic construct
  source 1..42: mol_type = other DNA
ggtcgactctagaggatcccccctggaagaagatctggtcgc

SEQ ID NO: 16 - DNA, 1134 bp, Corynebacterium glutamicum
  source 1..1134: mol_type = genomic DNA; note = metX
atgcccaccctcgcgccttcaggtcaacttgaaatccaagcgatcggtgatgtctccaccgaagccggagcaatcattacaaacgctgaaatcgcctatcaccgctggggtgaataccgcgtagataaagaaggacgcagcaatgtcgttctcatcgaacacgccctcactggagattccaacgcagccgattggtgggctgacttgctcggtcccggcaaagccatcaacactgatatttactgcgtgatctgtaccaacgtcatcggtggttgcaacggttccaccggacctggctccatgcatccagatggaaatttctggggtaatcgcttccccgccacgtccattcgtgatcaggtaaacgccgaaaaacaattcctcgacgcactcggcatcaccacggtcgccgcagtacttggtggttccatgggtggtgcccgcaccctagagtgggccgcaatgtacccagaaactgttggcgcagctgctgttcttgcagtttctgcacgcgccagcgcctggcaaatcggcattcaatccgcccaaattaaggcgattgaaaacgaccaccactggcacgaaggcaactactacgaatccggctgcaacccagccaccggactcggcgccgcccgacgcatcgcccacctcacctaccgtggcgaactagaaatcgacgaacgcttcggcaccaaagcccaaaagaacgaaaacccactcggtccctaccgcaagcccgaccagcgcttcgccgtggaatcctacttggactaccaagcagacaagctagtacagcgtttcgacgccggctcctacgtcttgctcaccgacgccctcaaccgccacgacattggtcgcgaccgcggaggcctcaacaaggcactcgaatccatcaaagttccagtccttgtcgcaggcgtagataccgatattttgtacccctaccaccagcaagaacacctctccagaaacctgggaaatctactggcaatggcaaaaatcgtatcccctgtcggccacgatgctttcctcaccgaaagccgccaaatggatcgcatcgtgaggaacttcttcagcctcatctccccagacgaagacaacccttcgacctacatcgagttctacatctaa

SEQ ID NO: 17 - DNA, 28 bp, synthetic construct
  source 1..28: mol_type = other DNA
ggatcccctcgttgttcacccagcaacc

SEQ ID NO: 18 - DNA, 30 bp, synthetic construct
  source 1..30: mol_type = other DNA
ggatcccaaagtcacaactacttatgttag

SEQ ID NO: 19 - DNA, 1314 bp, Corynebacterium glutamicum
  source 1..1314: mol_type = genomic DNA; note = metY
atgccaaagtacgacaattccaatgctgaccagtggggctttgaaacccgctccattcacgcaggccagtcagtagacgcacagaccagcgcacgaaaccttccgatctaccaatccaccgctttcgtgttcgactccgctgagcacgccaagcagcgtttcgcacttgaggatctaggccctgtttactcccgcctcaccaacccaaccgttgaggctttggaaaaccgcatcgcttccctcgaaggtggcgtccacgctgtagcgttctcctccggacaggccgcaaccaccaacgccattttgaacctggcaggagcgggcgaccacatcgtcacctccccacgcctctacggtggcaccgagactctattccttatcactcttaaccgcctgggtatcgatgtttccttcgtggaaaaccccgacgaccctgagtcctggcaggcagccgttcagccaaacaccaaagcattcttcggcgagactttcgccaacccacaggcagacgtcctggatattcctgcggtggctgaagttgcgcaccgcaacagcgttccactgatcatcgacaacaccatcgctaccgcagcgctcgtgcgcccgctcgagctcggcgcagacgttgtcgtcgcttccctcaccaagttctacaccggcaacggctccggactgggcggcgtgcttatcgacggcggaaagttcgattggactgtcgaaaaggatggaaagccagtattcccctacttcgtcactccagatgctgcttaccacggattgaagtacgcagaccttggtgcaccagccttcggcctcaaggttcgcgttggccttctacgcgacaccggctccaccctctccgcattcaacgcatgggctgcagtccagggcatcgacaccctttccctgcgcctggagcgccacaacgaaaacgccatcaaggttgcagaattcctcaacaaccacgagaaggtggaaaaggttaacttcgcaggcctgaaggattccccttggtacgcaaccaaggaaaagcttggcctgaagtacaccggctccgttctcaccttcgagatcaagggcggcaaggatgaggcttgggcatttatcgacgccctgaagctacactccaaccttgcaaacatcggcgatgttcgctccctcgttgttcacccagcaaccaccacccattcacagtccgacgaagctggcctggcacgcgcgggcgttacccagtccaccgtccgcctgtccgttggcatcgagaccattgatgatatcatcgctgacctcgaaggcggctttgctgcaatctag

SEQ ID NO: 20 - DNA, 18 bp, synthetic construct
  source 1..18: mol_type = other DNA
ccaaagacaaggagacca

SEQ ID NO: 21 - DNA, 40 bp, synthetic construct
  source 1..40: mol_type = other DNA
agtctatttaaagcccgggttggaggtccttaagagtttt

SEQ ID NO: 22 - DNA, 40 bp, synthetic construct
  source 1..40: mol_type = other DNA
taaggacctccaacccgggctttaaatagactcaccccag

SEQ ID NO: 23 - DNA, 18 bp, synthetic construct
  source 1..18: mol_type = other DNA
atgccgagtgcgtcgagg

SEQ ID NO: 24 - DNA, 1266 bp, Corynebacterium glutamicum
  source 1..1266: mol_type = genomic DNA; note = lysC
gtggccctggtcgtacagaaatatggcggttcctcgcttgagagtgcggaacgcattagaaacgtcgctgaacggatcgttgccaccaagaaggctggaaatgatgtcgtggttgtctgctccgcaatgggagacaccacggatgaacttctagaacttgcagcggcagtgaatcccgttccgccagctcgtgaaatggatatgctcctgactgctggtgagcgtatttctaacgctctcgtcgccatggctattgagtcccttggcgcagaagcccaatctttcacgggctctcaggctggtgtgctcaccaccgagcgccacggaaacgcacgcattgttgatgtcactccaggtcgtgtgcgtgaagcactcgatgagggcaagatctgcattgttgctggtttccagggtgttaataaagaaacccgcgatgtcaccacgttgggtcgtggtggttctgacaccactgcagttgcgttggcagctgctttgaacgctgatgtgtgtgagatttactcggacgttgacggtgtgtataccgctgacccgcgcatcgttcctaatgcacagaagctggaaaagctcagcttcgaagaaatgctggaacttgctgctgttggctccaagattttggtgctgcgcagtgttgaatacgctcgtgcattcaatgtgccacttcgcgtacgctcgtcttatagtaatgatcccggcactttgattgccggctctatggaggatattcctgtggaagaagcagtccttaccggtgtcgcaaccgacaagtccgaagccaaagtaaccgttctgggtatttccgataagccaggcgaggctgcgaaggttttccgtgcgttggctgatgcagaaatcaacattgacatggttctgcagaacgtctcttctgtagaagacggcaccaccgacatcaccttcacctgccctcgttccgacggccgccgcgcgatggagatcttgaagaagcttcaggttcagggcaactggaccaatgtgctttacgacgaccaggtcggcaaagtctccctcgtgggtgctggcatgaagtctcacccaggtgttaccgcagagttcatggaagctctgcgcgatgtcaacgtgaacatcgaattgatttccacctctgagattcgtatttccgtgctgatccgtgaagatgatctggatgctgctgcacgtgcattgcatgagcagttccagctgggcggcgaagacgaagccgtcgtttatgcaggcaccggacgctaa

SEQ ID NO: 25 - DNA, 19 bp, synthetic construct
  source 1..19: mol_type = other DNA
cagaagctggaaaagctca

SEQ ID NO: 26 - DNA, 40 bp, synthetic construct
  source 1..40: mol_type = other DNA
atctcagaggtggaaatcttttcgatgttcacgttgacat

SEQ ID NO: 27 - DNA, 40 bp, synthetic construct
  source 1..40: mol_type = other DNA
tgtcaacgtgaacatcgaaaagatttccacctctgagatt

SEQ ID NO: 28 - DNA, 19 bp, synthetic construct
  source 1..19: mol_type = other DNA
tccttgtcggaagggttca

SEQ ID NO: 29 - DNA, 777 bp, Corynebacterium glutamicum
  source 1..777: mol_type = genomic DNA; note = NCgl0616
atgagcgaacgtcagctggaaaagtcaattgagcacgccgtcgagttagcccgcgaagcccgaaacatcgaagtttttaccggagccggaatgagcgccgactccgggttggaaacgtatcgtgatgataaaaccgggctgtggagcaacgtagatccacaagcgatggcaagtatcgatgcatggcgcaaagatccagagccaatgtgggcgtggtatcgctggcgcgccggggtggcagctagggcagaacccaacgcggggcatcaagctatttcctactgggaggggagtgacaccgtcgaacacgttcacatcaccacccagaacattgacaacctgcacgagcgagctggctctagcgatgtgacacatcttcatggcagcttgtttgaatacaggtgctctgattgtgcgactccatgggaagacgataaaaactatccgcaagaacccattgcacgccttgctcctccacaatgtgaaaagtgcggagggctgattagaccaggtgtggtgtggtttggtgagaacctgcccgtagaagagtgggatattgcagagcaacgcatcgcagaagccgatctcatgatcattgtgggtacctccgggattgttcatcctgcagcagcactcccgcaattagcccaacaacgcggcgttcccatcgtggagatctccccaacgcgcaccgaacttagccggatcgcagacttcacctggatgtccaccgcagcccaagcgctaccagcgttgatgcgaggtttgagcgcctaa

SEQ ID NO: 30 - DNA, 36 bp, synthetic construct
  source 1..36: mol_type = other DNA
tcgagctcggtacccagcataattccatactcccac

SEQ ID NO: 31 - DNA, 42 bp, synthetic construct
  source 1..42: mol_type = other DNA
ggtagcgcttgggctgcagtactctcgacggcgtgctcaatt

SEQ ID NO: 32 - DNA, 42 bp, synthetic construct
  source 1..42: mol_type = other DNA
aattgagcacgccgtcgagagtactgcagcccaagcgctacc

SEQ ID NO: 33 - DNA, 34 bp, synthetic construct
  source 1..34: mol_type = other DNA
ctctagaggatccccctacgacgctactgcgcag

SEQ ID NO: 34 - DNA, 18 bp, synthetic construct
  source 1..18: mol_type = other DNA
ggcttccaactgtaatgg

SEQ ID NO: 35 - DNA, 18 bp, synthetic construct
  source 1..18: mol_type = other DNA
tagaacacccagctaaca